European Patent Application EP 4 144 847 A1, published March 8, 2023. Title: Microorganism expressing vasoactive intestinal peptide, and use thereof. Applicant: Medytox Inc. The sequence listing filed with the application follows.

SEQUENCE LISTING (34 sequences)

SEQ ID NO: 1 - protein, 28 aa, Homo sapiens
HSDAVFTDNYTRLRKQMAVKKYLNSILN

SEQ ID NO: 2 - protein, 28 aa, Artificial Sequence
  VIP variant 1
HSDAVFTDNYTRLRRQLAVRRYLNSILN

SEQ ID NO: 3 - protein, 30 aa, Artificial Sequence
  VIP variant 2
HSDAVFTANYTRLRRQLAVRRYLAAIGLRR

SEQ ID NO: 4 - protein, 25 aa, Artificial Sequence
  VIP variant 3
FTANYTRLRRQLAVRRYLAAILGRR

SEQ ID NO: 5 - protein, 28 aa, Artificial Sequence
  VIP variant 4
HSDGIFTDSYSRYRKQMAVKKYLAAVLN

SEQ ID NO: 6 - protein, 28 aa, Artificial Sequence
  VIP variant 5
HSDAVFTDNYARLRKQMAVKKALNSILA

SEQ ID NO: 7 - protein, 31 aa, Artificial Sequence
  VIP variant 6
HSDAVFTDNYTRLRKQVAAKKYLQSIKNKRY

SEQ ID NO: 8 - protein, 31 aa, Artificial Sequence
  VIP variant 7
HSDAVFTDNYTRLRRQLAVRRYLNSILNGRR

SEQ ID NO: 9 - protein, 23 aa, Artificial Sequence
  VIP variant 8
HSDAVFTDNYTRLRRQLAVRRYL

SEQ ID NO: 10 - DNA, 31 bp, Lactobacillus paracasei
tcgtcacggcgctgcttttttcatacaaaat

SEQ ID NO: 11 - DNA, 500 bp, Lactobacillus paracasei
tccacaatcaaggtgcttggctttttcgatcgcgaggtcaccatgtacatcagtcgtgagagcattgtgttgacagtgatcggcatcgtgttcggctatctgctcggcaatttgctgacagcctacattttgtatcaagccgaaactgaggccgtggtttttccactcacgatcagcattgtcggctacctcacggccacgttactcatgttggccttcaccggcgtcgtcacctggctcacgcatcgtcgactccaacgggtggacatggtcgaagccctgaaatcaaacgaataacctacaattttgtcaggcagcgtcgtcacggcgctgcttttttcatacaaaattcatcaaaaattgggattaaaaacgttcatgatcgcaattttgaagcgcaaatgaagattgagaccaactcctaacagtcctgtaacgctgacgtaacattgacacagtaaagtagcctttagttaatcaaattaagggtgaggtcaaaa

SEQ ID NO: 12 - protein, 31 aa, Lactobacillus paracasei
MKFNKVMITLVAAVTLAGSASAVTPVFADTS

SEQ ID NO: 13 - DNA, 93 bp, Lactobacillus paracasei
atgaaattcaataaagtcatgatcacgttggttgctgcagttaccttagcaggttctgctagcgccgtaacaccagttttcgctgatacaagc

SEQ ID NO: 14 - DNA, 1347 bp, Lactobacillus brevis
gtgatggataacaataataatcaatttaataaccaacaacatgatcataatgaagaaaccacaccaactccggaaccacggaaacggcggggtggcctgacactgacgaaagtggcagtgacggctgcggtcgctggactcttaggcggcggggttgcgtacggcggtatcaactactttaataatagtgggatgaatgatacggcggtgccagccgggagtaactcgaccgggaacaccaagacctctaacgtcaacgtcaatgtctcgagtcaatcaaccaaggcctttaataaggttaaaggggccatggtctcggtgattaatttacagaaggaaaatagtagtagcgggacgcttggccaattattcggctcaagctcgagctccaattcatcgaaatccaagtcagagctggaagaagcttccgaaggttctggggtgatttataagaaggacggtaacgtggcttacatcgtgacgaacaatcacgtggtttccggctcttcagccttacgagtcgtgacgagttccggtaaacaactgcaagcgaagttggttggtaaggattccgttaccgacttggccgtcttaaaggttaacggctcgtcattaaagaccgtggcgtcatttggaaactcagataatatcaaggttggggaaacggccttggcaattggctcaccactgggcagccaatacgcaacgtcattgacgcaagggatcatctccgccaagaagcggacgattgaaacgactaattcttcgggaacgcaaaccgggaatgcaacggttattcagacggatgcggcgattaaccctgggaactcagggggggccttgattaatgtcggtggccaagtggtcggcattacctcatcgaagatcgccagtgatgcggaaggcaccagcgttgaagggatgggctttgccattccatctaacgaagtggtcaatatcatcaatcaactggtcaagaacgggaaggtcgtgcggccagcgttagggattacctacgttgacttggcgaacgtttctagtgcgcaacagaaatcgatcctgaagttaccatctaatgtggaaaacggggtcgtggtgatgagtgcttcggcgggctcaccagcgaagaaggccggcttgagcaagtatgatgtgattacggcgctgggcggtcatcagatttcagaccaatccacgttgcgagatattttgtacaagtataagctgaacgataaggtctcgatcacttactatcacaatggtaagaagaagaccagcaccattaaattaacggaaacatcttctcaattaaagactagctcgacgacggcaacgtcagagagttag

SEQ ID NO: 15 - DNA, 2535 bp, Lactobacillus brevis
atgacagaatcaacgcacttgtatgacctgttccacccggcacactacgatatttatctcgatattaaccgcgaaacgaagcaaattagcgggaagacgacgattactggtgatgccttagccacgacgattggcattcaccagaagttcttaaagatccaacaggtaacggttgacggcaaagccgtgacggttacggatgatcctgcggccgaagccattcggattccggtcccacagacgggtaacgtgacgttagccattgattacacggcgccattaactgatagcatgatggggatttacccatcctactacgacgttaacggcgtacaaaagcaaatcattggaacccagtttgaaacgaccgctgcgcgccaagctttcccaagtatcgatgaaccggaggccaaagcaacctttgacctagcgattaagttcgatgaacagcctggtgaaacggttatcagtaacatgcctgagaccaaggtcgaagccggcgtgcactactttgacaccacggttaagatgtccacgtacctgattgcctttgcctttggtgatttgcaaagtaagatgacgactactaagagtggggttcaggttggggtgtttgctaccaaggcgcatcaagccaatgaattggactttgcgttagacattgccaagcgctcaattgaattttacgaagacttctatcagacaccttatccactaccacattcctggcagttagctttacctgacttttccgctggcgccatggaaaactggggattggttacttaccgggaagcttacctcgttttagaccccgacaatacgtcgtttgaaacgaagcaacgggttgccaccgtcattgctcatgaactggcccaccaatggtttggtgatttggttacgatgaagtggtgggatgatctttggttgaacgaaagttttgccaacatgatggaatacgttgctattgatgccatcgaacctgactggcacatttgggaagtcttccaaacaactgaagccccgatggccttacaacgggacgcaacggacggtgtacaatctgtccacgtgcaagtagaagatccagctgaaattgatgcgctctttgatagtgccattgtttacgccaagggtgcccggatgttagtcatggtacgggctttaattggcgatgatgctctgcgaacgggcctgaaggcttacttcgacgcccataagtttggtaatgcaactggggctgacttgtggtctgctttagggactgctgccaatatggatttgaagagcgtaatgaattcgtggctggaacaacctggttacccagtcttaacggctgcggtggtcgatggtcagttgacagtgacccagcaacaattctttattggcgatggcacagacgccaaacgtcaatggcaagtgccattgagcagtaactatgctgaagtcccagaattgttgacggcgccacaagtgacgttaggaacttatgcggatttacggcaggctaatggacagccgttccggctaaatgtcggcaataattcacatgcgattgtgaagtacgatgataccttactagcagatattttagatcacatcactgagttaacagcgattgatcaactccaattgctacaagatcaacgactactggctgaagggcggcagatttcttatgcggatgtcgtcgccttgttgccacgatttgcggctagtgaagctacggtggttaacgatgcgttgtatcaggtcgctggtaacttgaagaagttcgtcacgccagattctgatgccgaaaagcaactgcaacaattctttgatcggttaagtgcggcacaagttgaccggttggggtggacccctaaagctggcgaatctaatgatgaccagttaacccggccatatgtattaagcgcggccctctatgctaaaaatgcccaatcagtcgccgctgcgcatgaactgttcacagccaatcgcgacaatttagcaggcttgccagctgcaacgcgttactatgttttggcaaatgaagtcacgaacttcagtgacgcaacggtctttgatcagttgctgacagattaccggcaagcaacggatgccagctacaaggccgatctgtgtgccgcattgacgaccacaccagatgccaagttgattgcgaagttaatcgcagtctttgaaaacgcggccacggttaaaccacaggacttacgggcttggtaccgtggtgtcttggccaatgccaaggggcagcaggtggcttgggactggatccgtcaagattgggattggttggaagcaactgtgggtggtgatatggaattcaccacatttattacggtaactgcggcgatcttccacacacctgaacggttagctgagttcaaggaattctttgaaccaaagattccgacgcctggtttaggacgtgaaatcaagatggataccaaggttatcgcaagtcgcgtggccttagttgaagatgaaaaagccgcagtgaatgctgcggtggcacaagtcgtccaataa

SEQ ID NO: 16 - DNA, 597 bp, Lactobacillus brevis
atgaatttagtaccaacagttattgaacaatcatcccgtggcgaacgggcctatgatatttattcacgactattaaaagaccggattatcatgttatctggtccaattgaagatgacatggccaacgccatcatcgcgcagttactcttcttggatgcccaagactcaaccaaggacatttcactctacatcaactcacctggtggtgtcgtttcttccggcttggccatctatgataccatgaacttcatccaatctgacgtgcaaacgatcacgttagggatggcagcttccatggcaagtgtcttggcttcatctgggactaagggcaagcgttttgctttgcctcacgcccaagtgatgattcaccaaccatctggtggtgcccaaggacaacaaacggaaatcgaaattgctgctcgtgaaatcttgaagacccgtgaattgatcaacaagattttagcagagaattccggtcaaccgattgaacgcctcaatcaagatactgaacgagacaactacttgagtgctcaagaagcggttgattatggattaattgaccacatcatgaccaacagtagtgaacaaaagaagtaa

SEQ ID NO: 17 - DNA, 1050 bp, Lactobacillus brevis
gtgtggaatttaacgcgacggcagtggcggcagattctagtaacggtgatattagcacttgcagtgttgctattttttctgtggccattgcccaagtatattgagggtcccggtgaggcagacaatttgaaatcatttgtcacagttgcccaacatcccgataagcataagggaaaatatatgattacctcagttgcgttggcgcaagctcgtccagtttcctacctctatgccaaatttaatccctattacagcattgagagtgtagcgtcagtgacgggtggcgagagtaatgcgacctatgataaagttcagaacttttatatgaaaagcgccatcaatgagtcgatttataccgcatatcgggcggcccataaaacggtgaagcgtcattatttgggaatttacgttttgagtgttgatcgtcggtcaccctttgcccaagcgttaaaggtgggcgatacggtgacggaggtaaatggtcatcatttcaactctatgacggggtatcaacgatatatccagcgacaaaaagtgggacaacggacgaccattacgtatcagcacaatggtaaaacacaccacgtaactgccaaattgatgcggttgccaacgaaaaaagcgggtattgggattactttgacggataacgtcaaagttagtgctcggcctaaagtgcaggtgaatcccggcaacatcggtggtccgtcaggtggtttaatgtttagcttacagatttatacgcaagtgacggggcaggacttacgtcacgggcgaaagattgcaggaaccggaacggttgatggtgacggcaacgttggcgagattggtggtattgataagaaaattatcgctgctaagcgcgcaggggcgacggtcttctttgctccctacgtgaaaccgacaaaattgttactgaagtatgaagaacaacaccaaacgaattatcaattggctaaggcaacagcgaaaaagtatgcgccgaatatgaaagttgtgccagtaaaatcgtttgacgatgcagttcattacttaaggacacaccgttaa

SEQ ID NO: 18 - DNA, 606 bp, Lactobacillus brevis
atgttcacaggaataattacagatcaaggttacattcgacaaataaataaaacagccacgggagcacagctcgttattcaaacgacacgggctcatcagacacgacacgtcggggacagcatcgccgtgaacgggatctgcctcactttaaccgcagtgactgacgaagcatttaccgttgttgcaatggctgaaaccttgcagcgtacgacactgggaacttggcagactggtatgcaggtcaatctggaagctgctttacgagcagatcaaggattggatggacatatcgttcaggggcacgttgacaccacagcgaccttacgagcaagtcataccgaaggggccgcagtccggttgacctttgatgtatcagctgatcaagctccttacttggttgaaaagggtgctgtggccttggatggtgttagtttaacggtcacggcagttactcgtcagacggttcaggtagcgctgattccctatacgttggcacatacgagtcttggtcatctacagtgcggtgatcaggtgaatgtagagacagatattttggggaagtacgtggttcgtcagtaccagttaggggggatgactgatgactag

SEQ ID NO: 19 - DNA, 951 bp, Lactobacillus brevis
gatttgccggtgtccccggaattagcgaccaagtcccagtatagggcagtggaattacagtgagtagagtattagcttctatgagctgaatagtcctaaattggtgttgacaccgcgtcgtacaccacaggcgcgatcgacccaaaactaaacgagttgcactaatgacatttacacgcgcagtgggtcgcatacctgctttagcgggtggagattcgggtgaaggaatcgttagtcgctacagttgttacgcatcgaccgttataacttcccgtgtggatccttctatagtcgtgaagagaccatttcgactgtcgaattaaacggtagtaactgcattttaactttctcgcacaccgttccaccgtttcggtaactaccgtgtagtcggcctaaggtgcgactttgctagtaggcggctctcagacccacgcaggcgttgcagagttagtgtaaccggtcaactagttaccaaagtggaactactggaacggttcgggcggtgactgatggtatttgatctgggtttagtggtttcaccagtggttttcgaactaggcaatgctaagctagtgttttacggaaaaaaagacgaactataacgactaatttcagacgtaggtggttccttgccgctggtttcagccagtatagaccgggcactataagccctgatagttgcatcgcaactttccgggtgagcagggtttataccaacaccacaacgttatttttggcttataatcataggggtgcttccttggtgttctcaagcctaaattactctggtttcccgtggaaaaatcatcagttatcacccttcgggagaacgtttaatttggcgtaaaccatcggtttattcgattagcaaggccaagggcatgccaggcaaaaaagcactgggcagcagttctgtcagaatcgatttagatttatacggagaagattgtg

SEQ ID NO: 20 - DNA, 1818 bp, Lactobacillus brevis
atgtgtggaattgttggagtgacgggtaacgataacgccgttaaaattttagttaatgggctacaaaagttggaatatcgcggctatgattcagccggaatctatgttaatgaccaaaaaggccaggattatttggtaaaggccaagggccggatttccgaattaagtgctaagattacgccagaagttcacggatcaactgggattggtcatacgcgttgggcaacgcatggggtggttagcgtggataatgcgcacccacatttctccaacgacgaccgcttttacttggttcacaatggtgtgattgataacttccaagaacttaaggcgcaatatttaagtgatgtacctttccggagccaaacggatacagaagttgtcgtacagttgattgataagtttgcggtagaagatcacttagatgctaagcaggctttcttgaagacactaggcctgctgaagggttcctcatatgccttcttaatgatggatcgggaacaaccagacacattatttgtggctaagaacaagagccccttattaattggtgtcggcgatggcttcaacgttgtctgctcagatgccttggccatgttacgggaaacccacgatttcttggaattaatggatggtgaagttgtaacgatcacgccagataaagtggcaatcgaagacgctgatggtcagactgttgagcggaaacctttccacgttgacatgaacgctgatgaagcagacaagggcacttatccattctacatgttaaaagaagttgatgaacaacctaacgtgatgcgtaaattagcccaaacatatctgtcagaacacggcgaacctaacattgacaagcaattgctacaagcaatggaagccgctgatcgattgtatatcattggcgctgggacgagttaccacgctgggctgattggtaagcgcctctttgaaaacttggctcacattccaacggaagttcatgtgtcatcagaatttgcgtatgaacaaccgatgttatctgagaagccattctttattttcctgacccaatctggagaaacagctgatagtcgtgaagttttggttaacgtgaacgatgcgggttacccaagcttgacaatcaccaatgtgcaaaactccacgttatcacgtgaagccacttacaccttgttgttacatgccggtccagaaattgcggtggcttcaaccaaggcgtacacggcccaaattgctttggaagctatcttggccaaggctttaggtgaattaactggccagattattgcgcagaatttcaatattcggcaacagttgggactcgtcgcaactgggatgcaagccattgtggatgaaaaggataagctggaagaaatgtcttccaagtacttgttaaagactaaccgggcgttttacattggccgggggatcgaccacgccgtttccttagaagcagctttgaaactgaaagagatttcttatattcagtgtgaaggcttcgcgtctggtgaattaaagcatggcacgattgcattaattgaggctggaacaccagttattgggtttattacgcaggcgaagacggctggtttaacccggagtaacttacaagaaacgatggcccgtggtgcacaaacattgacgattgtccgggaaagtttagccgtagatggtgatgacttagtcttaccggatgtcgatgagatgttaatgccactcttaagtgttgtaccagcacaattgttggcctactacacgagtttaaataagggcttagatgttgataagccacggaacttggccaagagtgtgacagttgaataa

SEQ ID NO: 21 - DNA, 18 bp, Artificial Sequence
  primer
agcaacctttgacctagc

SEQ ID NO: 22 - DNA, 20 bp, Artificial Sequence
  primer
aattccatatcaccacccac

SEQ ID NO: 23 - DNA, 17 bp, Artificial Sequence
  primer
cccgatggccttacaac

SEQ ID NO: 24 - DNA, 18 bp, Artificial Sequence
  primer
ggaacggctgtccattag

SEQ ID NO: 25 - DNA, 20 bp, Artificial Sequence
  primer
ctaaatgaggagggttcgcg

SEQ ID NO: 26 - DNA, 19 bp, Artificial Sequence
  primer
aagctggcgctttcattcc

SEQ ID NO: 27 - DNA, 18 bp, Artificial Sequence
  primer
acctctaacgtcaacgtc

SEQ ID NO: 28 - DNA, 18 bp, Artificial Sequence
  primer
agttcccagggttaatcg

SEQ ID NO: 29 - DNA, 17 bp, Artificial Sequence
  primer
taaccgcagtgactgac

SEQ ID NO: 30 - DNA, 19 bp, Artificial Sequence
  primer
agctgatacatcaaaggtc

SEQ ID NO: 31 - DNA, 17 bp, Artificial Sequence
  primer
agcattgtgttatcagc

SEQ ID NO: 32 - DNA, 17 bp, Artificial Sequence
  primer
gcagcattggtagcaac

SEQ ID NO: 33 - DNA, 22 bp, Artificial Sequence
  primer
gtgtggcaaggtggcaaagcca

SEQ ID NO: 34 - DNA, 25 bp, Artificial Sequence
  primer
ccgatctacaggcccaactcgatga